European Patent Specification EP 4 326 898 B1, published July 31, 2024. Title: PROBES COMPRISING A SPLIT BARCODE REGION AND METHODS OF USE. Applicant: 10x Genomics, Inc. Application WO. The sequence listing filed with the application follows.

SEQUENCE LISTING (4 sequences)

SEQ ID NO: 1 - DNA, 50 bp, synthetic construct
  source 1..50: mol_type = other DNA
aactcacgacggtgtacacatgcgtctatttagtggagccataggcgtaa

SEQ ID NO: 2 - DNA, 50 bp, synthetic construct
  source 1..50: mol_type = other DNA
cgacgtatagtctacgagtttgcagtcacggggcctgaggtctcagtggc

SEQ ID NO: 3 - DNA, 50 bp, synthetic construct
  source 1..50: mol_type = other DNA
nnnnnnnnnnnnnnnnnnnntgcgtctatttagtggagcctgacccgtgc

SEQ ID NO: 4 - DNA, 50 bp, synthetic construct
  source 1..50: mol_type = other DNA
ccataggtattctacgagtttgcagtcacgnnnnnnnnnnnnnnnnnnnn